European Patent Application EP 4 148 062 A1, published March 15, 2023. Title: A promoter activated by the MYB47 and MYB95 proteins and the expression system. Applicant: Uniwersytet Jagielloñski Instytut Chemii Bioorganicznej Polskiej Akademii Nauk. The sequence listing filed with the application follows.

SEQUENCE LISTING (25 sequences)

SEQ ID NO: 1 - DNA, 36 bp, artificial
  pTSA1
gaatgaaatccacgtttaagttagttacaacggttt

SEQ ID NO: 2 - DNA, 1566 bp, artificial
  Prom35S:GFP-MYB47
atggtgagcaagggcgaggagctgttcaccggggtggtgcccatcctggtcgagctggacggcgacgtgaacggccacaagttcagcgtgtccggcgagggcgagggcgatgccacctacggcaagctgaccctgaagttcatctgcaccaccggcaagctgcccgtgccctggcccaccctcgtgaccaccttcacctacggcgtgcagtgcttcagccgctaccccgaccacatgaagcagcacgacttcttcaagtccgccatgcccgaaggctacgtccaggagcgcaccatcttcttcaaggacgacggcaactacaagacccgcgccgaggtgaagttcgagggcgacaccctggtgaaccgcatcgagctgaagggcatcgacttcaaggaggacggcaacatcctggggcacaagctggagtacaactacaacagccacaacgtctatatcatggccgacaagcagaagaacggcatcaaggtgaacttcaagatccgccacaacatcgaggacggcagcgtgcagctcgccgaccactaccagcagaacacccccatcggcgacggccccgtgctgctgcccgacaaccactacctgagcacccagtccgccctgagcaaagaccccaacgagaagcgcgatcacatggtcctgctggagttcgtgaccgccgccgggatcactcacggcatggacgagctgtacatcacaagtttgtacaaaaaagcaggctccgcggccgcccccttcaccatggggaggacgacatggttcgacgtcgacgggatgaagaaaggagagtggacggcagaggaagaccagaagctcggcgcttacatcaacgagcatggcgtttgtgattggcgttccctccccaaaagagctggtttgcagagatgtggaaagagctgcagattaaggtggcttaactatctaaagcctgggattagaagaggcaaattcactcctcaagaagaagaagaaatcatccaacttcatgctgttctcggaaacaggtgggcagccatggcgaagaagatgcagaatcgaacagacaatgatatcaagaaccattggaactcttgtctcaagaaaagactttcgagaaagggaatcgaccctatgacccacgagcccatcatcaaacacctcaccgtcaataccactaacgcagattgtggtaactcttccaccacgacgtccccgtcgacgacggaaagctctccttcctccggctcgtctcgtcttcttaacaaactcgccgcaggtatctcatctagacaacatagtctcgataggatcaagtacatcttgtcgaattcaataatcgaaagcagtgatcaagcaaaagaggaagaagaaaaagaagaagaagaagaagaaagagattcaatgatgggtcagaagattgacggtagtgaaggagaagatattcagatttggggcgaggaggaagttaggcgtttaatggagattgatgcaatggatatgtacgagatgacttcgtacgacgctgtcatgtacgagagtagtcacatacttgatcatctcttttga

SEQ ID NO: 3 - DNA, 1944 bp, artificial
  Prom35S:GFP-MYB95
tgagacttttcaacaaagggtaatatccggaaacctcctcggattccattgcccagctatctgtcactttattgtgaagatagtggaaaaggaaggtggctcctacaaatgccatcattgcgataaaggaaaggccatcgttgaagatgcctctgccgacagtggtcccaaagatggacccccacccacgaggagcatcgtggaaaaagaagacgttccaaccacgtcttcaaagcaagtggattgatgtgatatctccactgacgtaagggatgacgcacaatcccactatccttcgcaagacccttcctctatataaggaagttcatttcatttggagagaacacgggggactctagaggatccatggtgagcaagggcgaggagctgttcaccggggtggtgcccatcctggtcgagctggacggcgacgtgaacggccacaagttcagcgtgtccggcgagggcgagggcgatgccacctacggcaagctgaccctgaagttcatctgcaccaccggcaagctgcccgtgccctggcccaccctcgtgaccaccttcacctacggcgtgcagtgcttcagccgctaccccgaccacatgaagcagcacgacttcttcaagtccgccatgcccgaaggctacgtccaggagcgcaccatcttcttcaaggacgacggcaactacaagacccgcgccgaggtgaagttcgagggcgacaccctggtgaaccgcatcgagctgaagggcatcgacttcaaggaggacggcaacatcctggggcacaagctggagtacaactacaacagccacaacgtctatatcatggccgacaagcagaagaacggcatcaaggtgaacttcaagatccgccacaacatcgaggacggcagcgtgcagctcgccgaccactaccagcagaacacccccatcggcgacggccccgtgctgctgcccgacaaccactacctgagcacccagtccgccctgagcaaagaccccaacgagaagcgcgatcacatggtcctgctggagttcgtgaccgccgccgggatcactcacggcatggacgagctgtacatcacaagtttgtacaaaaaagcaggctccgcggccgcccccttcaccatggggaggacgacgtggttcgacgttgacgggttgaggaaaggagagtggacggcggaggaagaccggaagctcgtggtttacatcaacgaacacggtctaggcgagtggggttcactgcctaagagagccggtctacaaagatgtggaaagagttgtagattaagatggctgaattatttgaggcctgggattaaaagaggcaagttcactcctcaggaagaagaagaaatcatcaaataccatgctcttcttggaaacaggtgggcagcaatagctaagcaaatgccaaacagaacagataatgacataaagaaccattggaactcatgccttaagaaaagacttgctaaaaaaggaatcgatccaatgacccatgagccaacaacaacaacaagcctcaccgtcgatgtcacctcctcatcaactacgtcgtctcctacaccgagccctacttcttcttctttttcctcctgttcctctactggctctgcacgtttccttaacaagctcgctgctggaatctcgtcaagaaaacacggactagagagtatcaagacagtgatattggcagaacaaccaagagaagccgttgatgaagagaagatgatgacaattaacatgaaagagaaggaattgattagttgttacatggagattgatgagacgatgagtattgatgaactaccttgtgatgactcgacgtctggcttcgtggcttttgacgactactcattaatcgacccatacagagacggtgtgtacgtatctgatttctacgatgagactgaacaccttgacctgttccttctttga

SEQ ID NO: 4 - DNA, 2477 bp, artificial
  PromTSA1:GUS
aagcttgtctgtccatggattgatatccaaattcatgactagacagaattaacgcaaaaaatcgaaattccacaatattgacaaaatgaaatataaagtcattaatttttttagagttgtgagtttgtttttttacgtaataatagttttaaaaaatttaatttacataatagaaaactaataaaagtatttttactatgtcaaaaaatataagaaaacaaaccaacgtaacacataaaaaaatgagatgttcaaaaacgaatttgtacgagcttgaccacttaactattgagcaatctgatttgggaatggaaggcataaccaaaaaaaaaagagatgtgtttttaaaaaaattgactttattaaaataaatatttctatcttagttattccatcaatagttttttttttgttttttttcctatttccatgatattattattttcaataaaattataaaatgtcacatttactaatattaattatattatttcacatctagctgtttaacttttgctacacacaaaatgagttatctagaagaagagccacgagataaaagaatgaaatccacgtttaagttagttacaacggttttattttataagcgtatccatagctatgtgatgcttcttcaagctggatccccgggtggtcagtcccttatgttacgtcctgtagaaaccccaacccgtgaaatcaaaaaactcgacggcctgtgggcattcagtctggatcgcgaaaactgtggaattgatcagcgttggtgggaaagcgcgttacaagaaagccgggcaattgctgtgccaggcagttttaacgatcagttcgccgatgcagatattcgtaattatgcgggcaacgtctggtatcagcgcgaagtctttataccgaaaggttgggcaggccagcgtatcgtgctgcgtttcgatgcggtcactcattacggcaaagtgtgggtcaataatcaggaagtgatggagcatcagggcggctatacgccatttgaagccgatgtcacgccgtatgttattgccgggaaaagtgtacgtatcaccgtttgtgtgaacaacgaactgaactggcagactatcccgccgggaatggtgattaccgacgaaaacggcaagaaaaagcagtcttacttccatgatttctttaactatgccggaatccatcgcagcgtaatgctctacaccacgccgaacacctgggtggacgatatcaccgtggtgacgcatgtcgcgcaagactgtaaccacgcgtctgttgactggcaggtggtggccaatggtgatgtcagcgttgaactgcgtgatgcggatcaacaggtggttgcaactggacaaggcactagcgggactttgcaagtggtgaatccgcacctctggcaaccgggtgaaggttatctctatgaactgtgcgtcacagccaaaagccagacagagtgtgatatctacccgcttcgcgtcggcatccggtcagtggcagtgaagggcgaacagttcctgattaaccacaaaccgttctactttactggctttggtcgtcatgaagatgcggacttgcgtggcaaaggattcgataacgtgctgatggtgcacgaccacgcattaatggactggattggggccaactcctaccgtacctcgcattacccttacgctgaagagatgctcgactgggcagatgaacatggcatcgtggtgattgatgaaactgctgctgtcggctttaacctctctttaggcattggtttcgaagcgggcaacaagccgaaagaactgtacagcgaagaggcagtcaacggggaaactcagcaagcgcacttacaggcgattaaagagctgatagcgcgtgacaaaaaccacccaagcgtggtgatgtggagtattgccaacgaaccggatacccgtccgcaaggtgcacgggaatatttcgcgccactggcggaagcaacgcgtaaactcgacccgacgcgtccgatcacctgcgtcaatgtaatgttctgcgacgctcacaccgataccatcagcgatctctttgatgtgctgtgcctgaaccgttattacggatggtatgtccaaagcggcgatttggaaacggcagagaaggtactggaaaaagaacttctggcctggcaggagaaactgcatcagccgattatcatcaccgaatacggcgtggatacgttagccgggctgcactcaatgtacaccgacatgtggagtgaagagtatcagtgtgcatggctggatatgtatcaccgcgtctttgatcgcgtcagcgccgtcgtcggtgaacaggtatggaatttcgccgattttgcgacctcgcaaggcatattgcgcgttggcggtaacaagaaagggatcttcactcgcgaccgcaaaccgaagtcggcggcttttctgctgcaaaaacgctggactggcatgaacttcggtgaaaaaccgcagcagggaggcaaacaatga

SEQ ID NO: 5 - DNA, 804 bp, artificial
  MYB47_cDNA
atggggaggacgacatggttcgacgtcgacgggatgaagaaaggagagtggacggcagaggaagaccagaagctcggcgcttacatcaacgagcatggcgtttgtgattggcgttccctccccaaaagagctggtttgcagagatgtggaaagagctgcagattaaggtggcttaactatctaaagcctgggattagaagaggcaaattcactcctcaagaagaagaagaaatcatccaacttcatgctgttctcggaaacaggtgggcagccatggcgaagaagatgcagaatcgaacagacaatgatatcaagaaccattggaactcttgtctcaagaaaagactttcgagaaagggaatcgaccctatgacccacgagcccatcatcaaacacctcaccgtcaataccactaacgcagattgtggtaactcttccaccacgacgtccccgtcgacgacggaaagctctccttcctccggctcgtctcgtcttcttaacaaactcgccgcaggtatctcatctagacaacatagtctcgataggatcaagtacatcttgtcgaattcaataatcgaaagcagtgatcaagcaaaagaggaagaagaaaaagaagaagaagaagaagaaagagattcaatgatgggtcagaagattgacggtagtgaaggagaagatattcagatttggggcgaggaggaagttaggcgtttaatggagattgatgcaatggatatgtacgagatgacttcgtacgacgctgtcatgtacgagagtagtcacatacttgatcatctcttttga

SEQ ID NO: 6 - DNA, 816 bp, artificial
  MYB95_cDNA
atggggaggacgacgtggttcgacgttgacgggttgaggaaaggagagtggacggcggaggaagaccggaagctcgtggtttacatcaacgaacacggtctaggcgagtggggttcactgcctaagagagccggtctacaaagatgtggaaagagttgtagattaagatggctgaattatttgaggcctgggattaaaagaggcaagttcactcctcaggaagaagaagaaatcatcaaataccatgctcttcttggaaacaggtgggcagcaatagctaagcaaatgccaaacagaacagataatgacataaagaaccattggaactcatgccttaagaaaagacttgctaaaaaaggaatcgatccaatgacccatgagccaacaacaacaacaagcctcaccgtcgatgtcacctcctcatcaactacgtcgtctcctacaccgagccctacttcttcttctttttcctcctgttcctctactggctctgcacgtttccttaacaagctcgctgctggaatctcgtcaagaaaacacggactagagagtatcaagacagtgatattggcagaacaaccaagagaagccgttgatgaagagaagatgatgacaattaacatgaaagagaaggaattgattagttgttacatggagattgatgagacgatgagtattgatgaactaccttgtgatgactcgacgtctggcttcgtggcttttgacgactactcattaatcgacccatacagagacggtgtgtacgtatctgatttctacgatgagactgaacaccttgacctgttccttctttga

SEQ ID NO: 7 - protein, 267 aa, artificial
  MYB47_protein
MGRTTWFDVDGMKKGEWTAEEDQKLGAYINEHGVCDWRSLPKRAGLQRCGKSCRLRWLNYLKPGIRRGKFTPQEEEEIIQLHAVLGNRWAAMAKKMQNRTDNDIKNHWNSCLKKRLSRKGIDPMTHEPIIKHLTVNTTNADCGNSSTTTSPSTTESSPSSGSSRLLNKLAAGISSRQHSLDRIKYILSNSIIESSDQAKEEEEKEEEEEERDSMMGQKIDGSEGEDIQIWGEEEVRRLMEIDAMDMYEMTSYDAVMYESSHILDHLF

SEQ ID NO: 8 - protein, 271 aa, artificial
  MYB95_protein
MGRTTWFDVDGLRKGEWTAEEDRKLVVYINEHGLGEWGSLPKRAGLQRCGKSCRLRWLNYLRPGIKRGKFTPQEEEEIIKYHALLGNRWAAIAKQMPNRTDNDIKNHWNSCLKKRLAKKGIDPMTHEPTTTTSLTVDVTSSSTTSSPTPSPTSSSFSSCSSTGSARFLNKLAAGISSRKHGLESIKTVILAEQPREAVDEEKMMTINMKEKELISCYMEIDETMSIDELPCDDSTSGFVAFDDYSLIDPYRDGVYVSDFYDETEHLDLFLL

SEQ ID NO: 9 - DNA, 1566 bp, artificial; identical to SEQ ID NO: 2
  GFP-MYB47_cDNA

SEQ ID NO: 10 - DNA, 1578 bp, artificial
  GFP-MYB95_cDNA
atggtgagcaagggcgaggagctgttcaccggggtggtgcccatcctggtcgagctggacggcgacgtgaacggccacaagttcagcgtgtccggcgagggcgagggcgatgccacctacggcaagctgaccctgaagttcatctgcaccaccggcaagctgcccgtgccctggcccaccctcgtgaccaccttcacctacggcgtgcagtgcttcagccgctaccccgaccacatgaagcagcacgacttcttcaagtccgccatgcccgaaggctacgtccaggagcgcaccatcttcttcaaggacgacggcaactacaagacccgcgccgaggtgaagttcgagggcgacaccctggtgaaccgcatcgagctgaagggcatcgacttcaaggaggacggcaacatcctggggcacaagctggagtacaactacaacagccacaacgtctatatcatggccgacaagcagaagaacggcatcaaggtgaacttcaagatccgccacaacatcgaggacggcagcgtgcagctcgccgaccactaccagcagaacacccccatcggcgacggccccgtgctgctgcccgacaaccactacctgagcacccagtccgccctgagcaaagaccccaacgagaagcgcgatcacatggtcctgctggagttcgtgaccgccgccgggatcactcacggcatggacgagctgtacatcacaagtttgtacaaaaaagcaggctccgcggccgcccccttcaccatggggaggacgacgtggttcgacgttgacgggttgaggaaaggagagtggacggcggaggaagaccggaagctcgtggtttacatcaacgaacacggtctaggcgagtggggttcactgcctaagagagccggtctacaaagatgtggaaagagttgtagattaagatggctgaattatttgaggcctgggattaaaagaggcaagttcactcctcaggaagaagaagaaatcatcaaataccatgctcttcttggaaacaggtgggcagcaatagctaagcaaatgccaaacagaacagataatgacataaagaaccattggaactcatgccttaagaaaagacttgctaaaaaaggaatcgatccaatgacccatgagccaacaacaacaacaagcctcaccgtcgatgtcacctcctcatcaactacgtcgtctcctacaccgagccctacttcttcttctttttcctcctgttcctctactggctctgcacgtttccttaacaagctcgctgctggaatctcgtcaagaaaacacggactagagagtatcaagacagtgatattggcagaacaaccaagagaagccgttgatgaagagaagatgatgacaattaacatgaaagagaaggaattgattagttgttacatggagattgatgagacgatgagtattgatgaactaccttgtgatgactcgacgtctggcttcgtggcttttgacgactactcattaatcgacccatacagagacggtgtgtacgtatctgatttctacgatgagactgaacaccttgacctgttccttctttga

SEQ ID NO: 11 - protein, 521 aa, artificial
  GFP-MYB47_protein
MVSKGEELFTGVVPILVELDGDVNGHKFSVSGEGEGDATYGKLTLKFICTTGKLPVPWPTLVTTFTYGVQCFSRYPDHMKQHDFFKSAMPEGYVQERTIFFKDDGNYKTRAEVKFEGDTLVNRIELKGIDFKEDGNILGHKLEYNYNSHNVYIMADKQKNGIKVNFKIRHNIEDGSVQLADHYQQNTPIGDGPVLLPDNHYLSTQSALSKDPNEKRDHMVLLEFVTAAGITHGMDELYITSLYKKAGSAAAPFTMGRTTWFDVDGMKKGEWTAEEDQKLGAYINEHGVCDWRSLPKRAGLQRCGKSCRLRWLNYLKPGIRRGKFTPQEEEEIIQLHAVLGNRWAAMAKKMQNRTDNDIKNHWNSCLKKRLSRKGIDPMTHEPIIKHLTVNTTNADCGNSSTTTSPSTTESSPSSGSSRLLNKLAAGISSRQHSLDRIKYILSNSIIESSDQAKEEEEKEEEEEERDSMMGQKIDGSEGEDIQIWGEEEVRRLMEIDAMDMYEMTSYDAVMYESSHILDHLF

SEQ ID NO: 12 - protein, 525 aa, artificial
  GFP-MYB95_protein
MVSKGEELFTGVVPILVELDGDVNGHKFSVSGEGEGDATYGKLTLKFICTTGKLPVPWPTLVTTFTYGVQCFSRYPDHMKQHDFFKSAMPEGYVQERTIFFKDDGNYKTRAEVKFEGDTLVNRIELKGIDFKEDGNILGHKLEYNYNSHNVYIMADKQKNGIKVNFKIRHNIEDGSVQLADHYQQNTPIGDGPVLLPDNHYLSTQSALSKDPNEKRDHMVLLEFVTAAGITHGMDELYITSLYKKAGSAAAPFTMGRTTWFDVDGLRKGEWTAEEDRKLVVYINEHGLGEWGSLPKRAGLQRCGKSCRLRWLNYLRPGIKRGKFTPQEEEEIIKYHALLGNRWAAIAKQMPNRTDNDIKNHWNSCLKKRLAKKGIDPMTHEPTTTTSLTVDVTSSSTTSSPTPSPTSSSFSSCSSTGSARFLNKLAAGISSRKHGLESIKTVILAEQPREAVDEEKMMTINMKEKELISCYMEIDETMSIDELPCDDSTSGFVAFDDYSLIDPYRDGVYVSDFYDETEHLDLFLL

SEQ ID NO: 13 - DNA, 635 bp, artificial
  TSA1_promoter
gtctgtccatggattgatatccaaattcatgactagacagaattaacgcaaaaaatcgaaattccacaatattgacaaaatgaaatataaagtcattaatttttttagagttgtgagtttgtttttttacgtaataatagttttaaaaaatttaatttacataatagaaaactaataaaagtatttttactatgtcaaaaaatataagaaaacaaaccaacgtaacacataaaaaaatgagatgttcaaaaacgaatttgtacgagcttgaccacttaactattgagcaatctgatttgggaatggaaggcataaccaaaaaaaaaagagatgtgtttttaaaaaaattgactttattaaaataaatatttctatcttagttattccatcaatagttttttttttgttttttttcctatttccatgatattattattttcaataaaattataaaatgtcacatttactaatattaattatattatttcacatctagctgtttaacttttgctacacacaaaatgagttatctagaagaagagccacgagataaaagaatgaaatccacgtttaagttagttacaacggttttattttataagcgtatccatagctatgtgatgcttcttcaagct

SEQ ID NO: 14 - DNA, 30 bp, artificial
  pTSA1HindIIIF primer
agacaagcttgtctgtccatggattgatat

SEQ ID NO: 15 - DNA, 28 bp, artificial
  pTSA1BamHIR primer
acagggatccagcttgaagaagcatcac

SEQ ID NO: 16 - DNA, 36 bp, artificial
  mbox1-pTSA1-R primer
gaatgaaatctttccccaagttagttacaacggttt

SEQ ID NO: 17 - DNA, 36 bp, artificial
  mbox2-pTSA1-R primer
gaatgaaatccacgtttaacccctttacaacggttt

SEQ ID NO: 18 - DNA, 36 bp, artificial
  mbox1mbox2-pTSA1-R primer
aaaccgttgtaaaggggttggggaaagatttcattc

SEQ ID NO: 19 - DNA, 36 bp, artificial; identical to SEQ ID NO: 16
  mbox1-pTSA1-F primer

SEQ ID NO: 20 - DNA, 36 bp, artificial; identical to SEQ ID NO: 17
  mbox2-pTSA1-F primer

SEQ ID NO: 21 - DNA, 36 bp, artificial
  mbox1mbox 2-pTSA1-F
gaatgaaatctttccccaacccctttacaacggttt

SEQ ID NO: 22 - DNA, 36 bp, artificial; identical to SEQ ID NO: 1
  pTSA1-F

SEQ ID NO: 23 - DNA, 36 bp, artificial
  pTSA1-R
aaaccgttgtaactaacttaaacgtggatttcattc

SEQ ID NO: 24 - DNA, 8 bp, artificial
  box1
cacgttta

SEQ ID NO: 25 - DNA, 7 bp, artificial
  box2
gttagtt